European Patent Specification EP 3 824 900 B1, published May 20, 2026. Title: METHOD TO PREDICT RESPONSE TO PHARMACOLOGICAL CHAPERONE TREATMENT OF DISEASES. Applicant: AMICUS THERAPEUTICS, INC. Application EP. The sequence listing filed with the application follows.

SEQUENCE LISTING (566 sequences)

SEQ ID NO: 1 - protein, 398 aa, Homo sapiens
LDNGLARTPTMGWLHWERFMCNLDCQEEPDSCISEKLFMEMAELMVSEGWKDAGYEYLCIDDCWMAPQRDSEGRLQADPQRFPHGIRQLANYVHSKGLKLGIYADVGNKTCAGFPGSFGYYDIDAQTFADWGVDLLKFDGCYCDSLENLADGYKHMSLALNRTGRSIVYSCEWPLYMWPFQKPNYTEIRQYCNHWRNFADIDDSWKSIKSILDWTSFNQERIVDVAGPGGWNDPDMLVIGNFGLSWNQQVTQMALWAIMAAPLFMSNDLRHISPQAKALLQDKDVIAINQDPLGKQGYQLRQGDNFEVWERPLSGLAWAVAMINRQEIGGPRSYTIAVASLGKGVACNPACFITQLLPVKRKLGFYEWTSRLRSHINPTGTVLLQLENTMQMSLKDLL

SEQ ID NO: 2 - DNA, 1312 bp, Homo sapiens
gaattctccggtcaccgtgacaatgcagctgaggaacccagaactacatctgggctgcgcgcttgcgcttcgcttcctggccctcgtttcctgggacatccctggggctagagcactggacaatggattggcaaggacgcctaccatgggctggctgcactgggagcgcttcatgtgcaaccttgactgccaggaagagccagattcctgcatcagtgagaagctcttcatggagatggcagagctcatggtctcagaaggctggaaggatgcaggttatgagtacctctgcattgatgactgttggatggctccccaaagagattcagaaggcagacttcaggcagaccctcagcgctttcctcatgggattcgccagctagctaattatgttcacagcaaaggactgaagctagggatttatgcagatgttggaaataaaacctgcgcaggcttccctgggagttttggatactacgacattgatgcccagacctttgctgactggggagtagatctgctaaaatttgatggttgttactgtgacagtttggaaaatttggcagatggttataagcacatgtccttggccctgaataggactggcagaagcattgtgtactcctgtgagtggcctctttatatgtggccctttcaaaagcccaattatacagaaatccgacagtactgcaatcactggcgaaattttgctgacattgatgattcctggaaaagtataaagagtatcttggactggacatcttttaaccaggagagaattgttgatgttgctggaccagggggttggaatgacccagatatgttagtgattggcaactttggcctcagctggaatcagcaagtaactcagatggccctctgggctatcatggctgctcctttattcatgtctaatgacctccgacacatcagccctcaagccaaagctctccttcaggataaggacgtaattgccatcaatcaggaccccttgggcaagcaagggtaccagcttagacagggagacaactttgaagtgtgggaacgacctctctcaggcttagcctgggctgtagctatgataaaccggcaggagattggtggacctcgctcttataccatcgcagttgcttccctgggtaaaggagtggcctgtaatcctgcctgcttcatcacacagctcctccctgtgaaaaggaagctagggttctatgaatggacttcaaggttaagaagtcacataaatcccacaggcactgttttgcttcagctagaaaatacaatgcagatgtcattaaaagacttactttaa

SEQ ID NO: 3 - DNA, 3624 bp, Homo sapiens
cagttgggaaagctgaggttgtcgccggggccgcgggtggaggtcggggatgaggcagcaggtaggacagtgacctcggtgacgcgaaggaccccggccacctctaggttctcctcgtccgcccgttgttcagcgagggaggctctgggcctgccgcagctgacggggaaactgaggcacggagcgggcctgtaggagctgtccaggccatctccaaccatgggagtgaggcacccgccctgctcccaccggctcctggccgtctgcgccctcgtgtccttggcaaccgctgcactcctggggcacatcctactccatgatttcctgctggttccccgagagctgagtggctcctccccagtcctggaggagactcacccagctcaccagcagggagccagcagaccagggccccgggatgcccaggcacaccccggccgtcccagagcagtgcccacacagtgcgacgtcccccccaacagccgcttcgattgcgcccctgacaaggccatcacccaggaacagtgcgaggcccgcggctgctgctacatccctgcaaagcaggggctgcagggagcccagatggggcagccctggtgcttcttcccacccagctaccccagctacaagctggagaacctgagctcctctgaaatgggctacacggccaccctgacccgtaccacccccaccttcttccccaaggacatcctgaccctgcggctggacgtgatgatggagactgagaaccgcctccacttcacgatcaaagatccagctaacaggcgctacgaggtgcccttggagaccccgcgtgtccacagccgggcaccgtccccactctacagcgtggagttctccgaggagcccttcggggtgatcgtgcaccggcagctggacggccgcgtgctgctgaacacgacggtggcgcccctgttctttgcggaccagttccttcagctgtccacctcgctgccctcgcagtatatcacaggcctcgccgagcacctcagtcccctgatgctcagcaccagctggaccaggatcaccctgtggaaccgggaccttgcgcccacgcccggtgcgaacctctacgggtctcaccctttctacctggcgctggaggacggcgggtcggcacacggggtgttcctgctaaacagcaatgccatggatgtggtcctgcagccgagccctgcccttagctggaggtcgacaggtgggatcctggatgtctacatcttcctgggcccagagcccaagagcgtggtgcagcagtacctggacgttgtgggatacccgttcatgccgccatactggggcctgggcttccacctgtgccgctggggctactcctccaccgctatcacccgccaggtggtggagaacatgaccagggcccacttccccctggacgtccaatggaacgacctggactacatggactcccggagggacttcacgttcaacaaggatggcttccgggacttcccggccatggtgcaggagctgcaccagggcggccggcgctacatgatgatcgtggatcctgccatcagcagctcgggccctgccgggagctacaggccctacgacgagggtctgcggaggggggttttcatcaccaacgagaccggccagccgctgattgggaaggtatggcccgggtccactgccttccccgacttcaccaaccccacagccctggcctggtgggaggacatggtggctgagttccatgaccaggtgcccttcgacggcatgtggattgacatgaacgagccttccaacttcatcagaggctctgaggacggctgccccaacaatgagctggagaacccaccctacgtgcctggggtggttggggggaccctccaggcggccaccatctgtgcctccagccaccagtttctctccacacactacaacctgcacaacctctacggcctgaccgaagccatcgcctcccacagggcgctggtgaaggctcgggggacacgcccatttgtgatctcccgctcgacctttgctggccacggccgatacgccggccactggacgggggacgtgtggagctcctgggagcagctcgcctcctccgtgccagaaatcctgcagtttaacctgctgggggtgcctctggtcggggccgacgtctgcggcttcctgggcaacacctcagaggagctgtgtgtgcgctggacccagctgggggccttctaccccttcatgcggaaccacaacagcctgctcagtctgccccaggagccgtacagcttcagcgagccggcccagcaggccatgaggaaggccctcaccctgcgctacgcactcctcccccacctctacacactgttccaccaggcccacgtcgcgggggagaccgtggcccggcccctcttcctggagttccccaaggactctagcacctggactgtggaccaccagctcctgtggggggaggccctgctcatcaccccagtgctccaggccgggaaggccgaagtgactggctacttccccttgggcacatggtacgacctgcagacggtgccaatagaggcccttggcagcctcccacccccacctgcagctccccgtgagccagccatccacagcgaggggcagtgggtgacgctgccggcccccctggacaccatcaacgtccacctccgggctgggtacatcatccccctgcagggccctggcctcacaaccacagagtcccgccagcagcccatggccctggctgtggccctgaccaagggtggagaggcccgaggggagctgttctgggacgatggagagagcctggaagtgctggagcgaggggcctacacacaggtcatcttcctggccaggaataacacgatcgtgaatgagctggtacgtgtgaccagtgagggagctggcctgcagctgcagaaggtgactgtcctgggcgtggccacggcgccccagcaggtcctctccaacggtgtccctgtctccaacttcacctacagccccgacaccaaggtcctggacatctgtgtctcgctgttgatgggagagcagtttctcgtcagctggtgttagccgggcggagtgtgttagtctctccagagggaggctggttccccagggaagcagagcctgtgtgcgggcagcagctgtgtgcgggcctgggggttgcatgtgtcacctggagctgggcactaaccattccaagccgccgcatcgcttgtttccacctcctgggccggggctctggcccccaacgtgtctaggagagctttctccctagatcgcactgtgggccggggcctggagggctgctctgtgttaataagattgtaaggtttgccctcctcacctgttgccggcatgcgggtagtattagccacccccctccatctgttcccagcaccggagaagggggtgctcaggtggaggtgtggggtatgcacctgagctcctgcttcgcgcctgctgctctgccccaacgcgaccgcttcccggctgcccagagggctggatgcctgccggtccccgagcaagcctgggaactcaggaaaattcacaggacttgggagattctaaatcttaagtgcaattattttaataaaaggggcatttggaatc

SEQ ID NO: 4 - protein, 952 aa, Homo sapiens
MGVRHPPCSHRLLAVCALVSLATAALLGHILLHDFLLVPRELSGSSPVLEETHPAHQQGASRPGPRDAQAHPGRPRAVPTQCDVPPNSRFDCAPDKAITQEQCEARGCCYIPAKQGLQGAQMGQPWCFFPPSYPSYKLENLSSSEMGYTATLTRTTPTFFPKDILTLRLDVMMETENRLHFTIKDPANRRYEVPLETPRVHSRAPSPLYSVEFSEEPFGVIVHRQLDGRVLLNTTVAPLFFADQFLQLSTSLPSQYITGLAEHLSPLMLSTSWTRITLWNRDLAPTPGANLYGSHPFYLALEDGGSAHGVFLLNSNAMDVVLQPSPALSWRSTGGILDVYIFLGPEPKSVVQQYLDVVGYPFMPPYWGLGFHLCRWGYSSTAITRQVVENMTRAHFPLDVQWNDLDYMDSRRDFTFNKDGFRDFPAMVQELHQGGRRYMMIVDPAISSSGPAGSYRPYDEGLRRGVFITNETGQPLIGKVWPGSTAFPDFTNPTALAWWEDMVAEFHDQVPFDGMWIDMNEPSNFIRGSEDGCPNNELENPPYVPGVVGGTLQAATICASSHQFLSTHYNLHNLYGLTEAIASHRALVKARGTRPFVISRSTFAGHGRYAGHWTGDVWSSWEQLASSVPEILQFNLLGVPLVGADVCGFLGNTSEELCVRWTQLGAFYPFMRNHNSLLSLPQEPYSFSEPAQQAMRKALTLRYALLPHLYTLFHQAHVAGETVARPLFLEFPKDSSTWTVDHQLLWGEALLITPVLQAGKAEVTGYFPLGTWYDLQTVPIEALGSLPPPPAAPREPAIHSEGQWVTLPAPLDTINVHLRAGYIIPLQGPGLTTTESRQQPMALAVALTKGGEARGELFWDDGESLEVLERGAYTQVIFLARNNTIVNELVRVTSEGAGLQLQKVTVLGVATAPQQVLSNGVPVSNFTYSPDTKVLDICVSLLMGEQFLVSWC

SEQ ID NO: 5 - DNA, 18 bp, Artificial Sequence
  Synthetic oligonucleotide
cgtgacaatacagctgag

SEQ ID NO: 6 - DNA, 18 bp, Artificial Sequence
  Synthetic oligonucleotide
ctcagctgtattgtcacg

SEQ ID NO: 7 - DNA, 22 bp, Artificial Sequence
  Synthetic oligonucleotide
caccgtgacaacgcagctgagg

SEQ ID NO: 8 - DNA, 22 bp, Artificial Sequence
  Synthetic oligonucleotide
cctcagctgcgttgtcacggtg

SEQ ID NO: 9 - DNA, 20 bp, Artificial Sequence
  Synthetic oligonucleotide
ggctgcgcgcctgcgcttcg

SEQ ID NO: 10 - DNA, 20 bp, Artificial Sequence
  Synthetic oligonucleotide
cgaagcgcaggcgcgcagcc

SEQ ID NO: 11 - DNA, 22 bp, Artificial Sequence
  Synthetic oligonucleotide
gcgcttgcgcmtcgcttcctgg

SEQ ID NO: 12 - DNA, 22 bp, Artificial Sequence
  Synthetic oligonucleotide
ccaggaagcgakgcgcaagcgc

SEQ ID NO: 13 - DNA, 24 bp, Artificial Sequence
  Synthetic oligonucleotide
gcttcgcttcccggccctcgtttc

SEQ ID NO: 14 - DNA, 24 bp, Artificial Sequence
  Synthetic oligonucleotide
gaaacgagggccgggaagcgaagc

SEQ ID NO: 15 - DNA, 23 bp, Artificial Sequence
  Synthetic oligonucleotide
ggggctagagtactggacaatgg

SEQ ID NO: 16 - DNA, 23 bp, Artificial Sequence
  Synthetic oligonucleotide
ccattgtccagtactctagcccc

SEQ ID NO: 17 - DNA, 21 bp, Artificial Sequence
  Synthetic oligonucleotide
gctagagcaccggacaatgga

SEQ ID NO: 18 - DNA, 21 bp, Artificial Sequence
  Synthetic oligonucleotide
tccattgtccggtgctctagc

SEQ ID NO: 19 - DNA, 21 bp, Artificial Sequence
  Synthetic oligonucleotide
gctagagcaccggacaatgga

SEQ ID NO: 20 - DNA, 21 bp, Artificial Sequence
  Synthetic oligonucleotide
tccattgtccggtgctctagc

SEQ ID NO: 21 - DNA, 23 bp, Artificial Sequence
  Synthetic oligonucleotide
ctagagcactgtacaatggattg

SEQ ID NO: 22 - DNA, 23 bp, Artificial Sequence
  Synthetic oligonucleotide
caatccattgtacagtgctctag

SEQ ID NO: 23 - DNA, 20 bp, Artificial Sequence
  Synthetic oligonucleotide
gcactggacaaaggattggc

SEQ ID NO: 24 - DNA, 20 bp, Artificial Sequence
  Synthetic oligonucleotide
gccaatcctttgtccagtgc

SEQ ID NO: 25 - DNA, 20 bp, Artificial Sequence
  Synthetic oligonucleotide
gcactggacagtggattggc

SEQ ID NO: 26 - DNA, 20 bp, Artificial Sequence
  Synthetic oligonucleotide
gccaatccactgtccagtgc

SEQ ID NO: 27 - DNA, 21 bp, Artificial Sequence
  Synthetic oligonucleotide
ctggacaatagattggcaagg

SEQ ID NO: 28 - DNA, 26 bp, Artificial Sequence
  Synthetic oligonucleotide
gtcagcaaaattttgccagtgattgc

SEQ ID NO: 29 - DNA, 23 bp, Artificial Sequence
  Synthetic oligonucleotide
gcgaaattttactgacattgatg

SEQ ID NO: 30 - DNA, 23 bp, Artificial Sequence
  Synthetic oligonucleotide
catcaatgtcagtaaaatttcgc

SEQ ID NO: 31 - DNA, 31 bp, Artificial Sequence
  Synthetic oligonucleotide
ggcgaaattttgctaacattgatgattcctg

SEQ ID NO: 32 - DNA, 31 bp, Artificial Sequence
  Synthetic oligonucleotide
caggaatcatcaatgttagcaaaatttcgcc

SEQ ID NO: 33 - DNA, 28 bp, Artificial Sequence
  Synthetic oligonucleotide
cgaaattttgctggcattgatgatattc

SEQ ID NO: 34 - DNA, 28 bp, Artificial Sequence
  Synthetic oligonucleotide
gaatatcatcaatgccagcaaaatttcg

SEQ ID NO: 35 - DNA, 24 bp, Artificial Sequence
  Synthetic oligonucleotide
tgacattgatgagtcctggaaaag

SEQ ID NO: 36 - DNA, 24 bp, Artificial Sequence
  Synthetic oligonucleotide
cttttccaggactcatcaatgtca

SEQ ID NO: 37 - DNA, 26 bp, Artificial Sequence
  Synthetic oligonucleotide
gctgacattgattattcctggaaaag

SEQ ID NO: 38 - DNA, 26 bp, Artificial Sequence
  Synthetic oligonucleotide
cttttccaggaataatcaatgtcagc

SEQ ID NO: 39 - DNA, 34 bp, Artificial Sequence
  Synthetic oligonucleotide
ctgacattgatgattgctggaaaagtataaagag

SEQ ID NO: 40 - DNA, 34 bp, Artificial Sequence
  Synthetic oligonucleotide
ctctttatacttttccagcaatcatcaatgtcag

SEQ ID NO: 41 - DNA, 39 bp, Artificial Sequence
  Synthetic oligonucleotide
gctgacattgatgattcccggaaaagtataaagagtatc

SEQ ID NO: 42 - DNA, 39 bp, Artificial Sequence
  Synthetic oligonucleotide
gatactctttatacttttccgggaatcatcaatgtcagc

SEQ ID NO: 43 - DNA, 23 bp, Artificial Sequence
  Synthetic oligonucleotide
tgatgattccttgaaaagtataa

SEQ ID NO: 44 - DNA, 23 bp, Artificial Sequence
  Synthetic oligonucleotide
ttatacttttcaaggaatcatca

SEQ ID NO: 45 - DNA, 34 bp, Artificial Sequence
  Synthetic oligonucleotide
ctgacattgatgattccttgaaaagtataaagag

SEQ ID NO: 46 - DNA, 34 bp, Artificial Sequence
  Synthetic oligonucleotide
ctctttatacttttcaaggaatcatcaatgtcag

SEQ ID NO: 47 - DNA, 43 bp, Artificial Sequence
  Synthetic oligonucleotide
gctgacattgatgattcctgtaaaagtataaagagtatcttgg

SEQ ID NO: 48 - DNA, 43 bp, Artificial Sequence
  Synthetic oligonucleotide
ccaagatactctttatacttttacaggaatcatcaatgtcagc

SEQ ID NO: 49 - DNA, 21 bp, Artificial Sequence
  Synthetic oligonucleotide
tggaaaagtacaaagagtatc

SEQ ID NO: 50 - DNA, 21 bp, Artificial Sequence
  Synthetic oligonucleotide
gatactctttgtacttttcca

SEQ ID NO: 51 - DNA, 21 bp, Artificial Sequence
  Synthetic oligonucleotide
ccttgccaatctattgtccag

SEQ ID NO: 52 - DNA, 20 bp, Artificial Sequence
  Synthetic oligonucleotide
aatggattggtaaggacgcc

SEQ ID NO: 53 - DNA, 20 bp, Artificial Sequence
  Synthetic oligonucleotide
ggcgtccttaccaatccatt

SEQ ID NO: 54 - DNA, 20 bp, Artificial Sequence
  Synthetic oligonucleotide
gcaaggacgcttaccatggg

SEQ ID NO: 55 - DNA, 20 bp, Artificial Sequence
  Synthetic oligonucleotide
cccatggtaagcgtccttgc

SEQ ID NO: 56 - DNA, 20 bp, Artificial Sequence
  Synthetic oligonucleotide
gcaaggacgtctaccatggg

SEQ ID NO: 57 - DNA, 20 bp, Artificial Sequence
  Synthetic oligonucleotide
cccatggtagacgtccttgc

SEQ ID NO: 58 - DNA, 27 bp, Artificial Sequence
  Synthetic oligonucleotide
aggacgcctaccacgggctggctgcac

SEQ ID NO: 59 - DNA, 27 bp, Artificial Sequence
  Synthetic oligonucleotide
gtgcagccagcccgtggtaggcgtcct

SEQ ID NO: 60 - DNA, 27 bp, Artificial Sequence
  Synthetic oligonucleotide
aggacgcctaccttgggctggctgcac

SEQ ID NO: 61 - DNA, 27 bp, Artificial Sequence
  Synthetic oligonucleotide
gtgcagccagcccaaggtaggcgtcct

SEQ ID NO: 62 - DNA, 25 bp, Artificial Sequence
  Synthetic oligonucleotide
aggacgcctaccgtgggctggctgc

SEQ ID NO: 63 - DNA, 25 bp, Artificial Sequence
  Synthetic oligonucleotide
gcagccagcccacggtaggcgtcct

SEQ ID NO: 64 - DNA, 20 bp, Artificial Sequence
  Synthetic oligonucleotide
ctaccatggwctggctgcac

SEQ ID NO: 65 - DNA, 20 bp, Artificial Sequence
  Synthetic oligonucleotide
gtgcagccagwccatggtag

SEQ ID NO: 66 - DNA, 20 bp, Artificial Sequence
  Synthetic oligonucleotide
ctaccatgcgctggctgcac

SEQ ID NO: 67 - DNA, 20 bp, Artificial Sequence
  Synthetic oligonucleotide
gtgcagccagcgcatggtag

SEQ ID NO: 68 - DNA, 19 bp, Artificial Sequence
  Synthetic oligonucleotide
catgggctgtctgcactgg

SEQ ID NO: 69 - DNA, 19 bp, Artificial Sequence
  Synthetic oligonucleotide
ccagtgcagacagcccatg

SEQ ID NO: 70 - DNA, 21 bp, Artificial Sequence
  Synthetic oligonucleotide
atgggctggcggcactgggag

SEQ ID NO: 71 - DNA, 21 bp, Artificial Sequence
  Synthetic oligonucleotide
ctcccagtgccgccagcccat

SEQ ID NO: 72 - DNA, 17 bp, Artificial Sequence
  Synthetic oligonucleotide
ctggctgcgctgggagc

SEQ ID NO: 73 - DNA, 17 bp, Artificial Sequence
  Synthetic oligonucleotide
gctcccagcgcagccag

SEQ ID NO: 74 - DNA, 17 bp, Artificial Sequence
  Synthetic oligonucleotide
ctggctgtactgggagc

SEQ ID NO: 75 - DNA, 17 bp, Artificial Sequence
  Synthetic oligonucleotide
gctcccagtacagccag

SEQ ID NO: 76 - DNA, 35 bp, Artificial Sequence
  Synthetic oligonucleotide
gattcctggaaaagtacaaagagtatcttggactg

SEQ ID NO: 77 - DNA, 35 bp, Artificial Sequence
  Synthetic oligonucleotide
cagtccaagatactctttgtacttttccaggaatc

SEQ ID NO: 78 - DNA, 26 bp, Artificial Sequence
  Synthetic oligonucleotide
agtataaagagtttcttggactggac

SEQ ID NO: 79 - DNA, 26 bp, Artificial Sequence
  Synthetic oligonucleotide
gtccagtccaagaaactctttatact

SEQ ID NO: 80 - DNA, 23 bp, Artificial Sequence
  Synthetic oligonucleotide
gtataaagagtaacttggactgg

SEQ ID NO: 81 - DNA, 23 bp, Artificial Sequence
  Synthetic oligonucleotide
ccagtccaagttactctttatac

SEQ ID NO: 82 - DNA, 22 bp, Artificial Sequence
  Synthetic oligonucleotide
agagtatcttcgactggacatc

SEQ ID NO: 83 - DNA, 22 bp, Artificial Sequence
  Synthetic oligonucleotide
gatgtccagtcgaagatactct

SEQ ID NO: 84 - DNA, 21 bp, Artificial Sequence
  Synthetic oligonucleotide
gagtatcttgcactggacatc

SEQ ID NO: 85 - DNA, 22 bp, Artificial Sequence
  Synthetic oligonucleotide
gatgtccagtcgaagatactct

SEQ ID NO: 86 - DNA, 30 bp, Artificial Sequence
  Synthetic oligonucleotide
cttggactggacatgttttaaccaggagag

SEQ ID NO: 87 - DNA, 30 bp, Artificial Sequence
  Synthetic oligonucleotide
ctctcctggttaaaacatgtccagtccaag

SEQ ID NO: 88 - DNA, 21 bp, Artificial Sequence
  Synthetic oligonucleotide
ggactggacaccttttaacca

SEQ ID NO: 89 - DNA, 21 bp, Artificial Sequence
  Synthetic oligonucleotide
tggttaaaaggtgtccagtcc

SEQ ID NO: 90 - DNA, 19 bp, Artificial Sequence
  Synthetic oligonucleotide
gttgatgttcctggaccag

SEQ ID NO: 91 - DNA, 19 bp, Artificial Sequence
  Synthetic oligonucleotide
ctggtccaggaacatcaac

SEQ ID NO: 92 - DNA, 19 bp, Artificial Sequence
  Synthetic oligonucleotide
gatgttgctcgaccagggg

SEQ ID NO: 93 - DNA, 19 bp, Artificial Sequence
  Synthetic oligonucleotide
cccctggtcgagcaacatc

SEQ ID NO: 94 - DNA, 25 bp, Artificial Sequence
  Synthetic oligonucleotide
gatgttgctggacgagggggttgga

SEQ ID NO: 95 - DNA, 25 bp, Artificial Sequence
  Synthetic oligonucleotide
tccaaccccctcgtccagcaacatc

SEQ ID NO: 96 - DNA, 21 bp, Artificial Sequence
  Synthetic oligonucleotide
gttgctggactagggggttgg

SEQ ID NO: 97 - DNA, 21 bp, Artificial Sequence
  Synthetic oligonucleotide
ccaaccccctagtccagcaac

SEQ ID NO: 98 - DNA, 22 bp, Artificial Sequence
  Synthetic oligonucleotide
gctggaccagcgggttggaatg

SEQ ID NO: 99 - DNA, 22 bp, Artificial Sequence
  Synthetic oligonucleotide
cattccaacccgctggtccagc

SEQ ID NO: 100 - DNA, 21 bp, Artificial Sequence
  Synthetic oligonucleotide
ggaccaggggattggaatgac

SEQ ID NO: 101 - DNA, 22 bp, Artificial Sequence
  Synthetic oligonucleotide
ctggctgcacggggagcgcttc

SEQ ID NO: 102 - DNA, 22 bp, Artificial Sequence
  Synthetic oligonucleotide
gaagcgctccccgtgcagccag

SEQ ID NO: 103 - DNA, 22 bp, Artificial Sequence
  Synthetic oligonucleotide
ctggctgcacttggagcgcttc

SEQ ID NO: 104 - DNA, 22 bp, Artificial Sequence
  Synthetic oligonucleotide
gaagcgctccaagtgcagccag

SEQ ID NO: 105 - DNA, 22 bp, Artificial Sequence
  Synthetic oligonucleotide
gctgcactggaagcgcttcatg

SEQ ID NO: 106 - DNA, 22 bp, Artificial Sequence
  Synthetic oligonucleotide
catgaagcgcttccagtgcagc

SEQ ID NO: 107 - DNA, 20 bp, Artificial Sequence
  Synthetic oligonucleotide
actgggagcycttcatgtgc

SEQ ID NO: 108 - DNA, 20 bp, Artificial Sequence
  Synthetic oligonucleotide
gcacatgaagrgctcccagt

SEQ ID NO: 109 - DNA, 19 bp, Artificial Sequence
  Synthetic oligonucleotide
cactgggagrgcttcatgt

SEQ ID NO: 110 - DNA, 19 bp, Artificial Sequence
  Synthetic oligonucleotide
acatgaagcyctcccagtg

SEQ ID NO: 111 - DNA, 22 bp, Artificial Sequence
  Synthetic oligonucleotide
ctgggagcgctgcatgtgcaac

SEQ ID NO: 112 - DNA, 22 bp, Artificial Sequence
  Synthetic oligonucleotide
gttgcacatgcagcgctcccag

SEQ ID NO: 113 - DNA, 22 bp, Artificial Sequence
  Synthetic oligonucleotide
gagcgcttcaagtgcaaccttg

SEQ ID NO: 114 - DNA, 22 bp, Artificial Sequence
  Synthetic oligonucleotide
caaggttgcacttgaagcgctc

SEQ ID NO: 115 - DNA, 17 bp, Artificial Sequence
  Synthetic oligonucleotide
gcgcttcatatgcaacc

SEQ ID NO: 116 - DNA, 17 bp, Artificial Sequence
  Synthetic oligonucleotide
ggttgcatatgaagcgc

SEQ ID NO: 117 - DNA, 26 bp, Artificial Sequence
  Synthetic oligonucleotide
gagcgcttcatgtccaaccttgactg

SEQ ID NO: 118 - DNA, 26 bp, Artificial Sequence
  Synthetic oligonucleotide
cagtcaaggttggacatgaagcgctc

SEQ ID NO: 119 - DNA, 21 bp, Artificial Sequence
  Synthetic oligonucleotide
cgcttcatgsgcaaccttgac

SEQ ID NO: 120 - DNA, 21 bp, Artificial Sequence
  Synthetic oligonucleotide
gtcaaggttgcscatgaagcg

SEQ ID NO: 121 - DNA, 20 bp, Artificial Sequence
  Synthetic oligonucleotide
caaccttgacggccaggaag

SEQ ID NO: 122 - DNA, 20 bp, Artificial Sequence
  Synthetic oligonucleotide
cttcctggccgtcaaggttg

SEQ ID NO: 123 - DNA, 22 bp, Artificial Sequence
  Synthetic oligonucleotide
caaccttgactwccaggaagag

SEQ ID NO: 124 - DNA, 22 bp, Artificial Sequence
  Synthetic oligonucleotide
ctcttcctggwagtcaaggttg

SEQ ID NO: 125 - DNA, 29 bp, Artificial Sequence
  Synthetic oligonucleotide
gtgcaaccttgactaccaggaagagccag

SEQ ID NO: 126 - DNA, 21 bp, Artificial Sequence
  Synthetic oligonucleotide
gtcattccaatcccctggtcc

SEQ ID NO: 127 - DNA, 21 bp, Artificial Sequence
  Synthetic oligonucleotide
cagggggttgcaatgacccag

SEQ ID NO: 128 - DNA, 21 bp, Artificial Sequence
  Synthetic oligonucleotide
ctgggtcattgcaaccccctg

SEQ ID NO: 129 - DNA, 19 bp, Artificial Sequence
  Synthetic oligonucleotide
ggggttggagtgacccaga

SEQ ID NO: 130 - DNA, 19 bp, Artificial Sequence
  Synthetic oligonucleotide
tctgggtcactccaacccc

SEQ ID NO: 131 - DNA, 21 bp, Artificial Sequence
  Synthetic oligonucleotide
ggttggaatgtcccagatatg

SEQ ID NO: 132 - DNA, 21 bp, Artificial Sequence
  Synthetic oligonucleotide
catatctgggacattccaacc

SEQ ID NO: 133 - DNA, 22 bp, Artificial Sequence
  Synthetic oligonucleotide
gggttggaattacccagatatg

SEQ ID NO: 134 - DNA, 22 bp, Artificial Sequence
  Synthetic oligonucleotide
catatctgggtaattccaaccc

SEQ ID NO: 135 - DNA, 21 bp, Artificial Sequence
  Synthetic oligonucleotide
tggaatgaccgagatatgtta

SEQ ID NO: 136 - DNA, 21 bp, Artificial Sequence
  Synthetic oligonucleotide
taacatatctcggtcattcca

SEQ ID NO: 137 - DNA, 23 bp, Artificial Sequence
  Synthetic oligonucleotide
ttggaatgacctagatatgttag

SEQ ID NO: 138 - DNA, 23 bp, Artificial Sequence
  Synthetic oligonucleotide
ctaacatatctaggtcattccaa

SEQ ID NO: 139 - DNA, 23 bp, Artificial Sequence
  Synthetic oligonucleotide
ggaatgacccamatatgttagtg

SEQ ID NO: 140 - DNA, 22 bp, Artificial Sequence
  Synthetic oligonucleotide
cactaacatattgggtcattcc

SEQ ID NO: 141 - DNA, 32 bp, Artificial Sequence
  Synthetic oligonucleotide
ggttggaatgacccacatatgttagtgattgg

SEQ ID NO: 142 - DNA, 32 bp, Artificial Sequence
  Synthetic oligonucleotide
ccaatcactaacatatgtgggtcattccaacc

SEQ ID NO: 143 - DNA, 22 bp, Artificial Sequence
  Synthetic oligonucleotide
gaatgacccagttatgttagtg

SEQ ID NO: 144 - DNA, 22 bp, Artificial Sequence
  Synthetic oligonucleotide
cactaacataactgggtcattc

SEQ ID NO: 145 - DNA, 21 bp, Artificial Sequence
  Synthetic oligonucleotide
atgacccagaaatgttagtga

SEQ ID NO: 146 - DNA, 21 bp, Artificial Sequence
  Synthetic oligonucleotide
tcactaacatttctgggtcat

SEQ ID NO: 147 - DNA, 22 bp, Artificial Sequence
  Synthetic oligonucleotide
gacccagataggttagtgattg

SEQ ID NO: 148 - DNA, 22 bp, Artificial Sequence
  Synthetic oligonucleotide
caatcactaacctatctgggtc

SEQ ID NO: 149 - DNA, 23 bp, Artificial Sequence
  Synthetic oligonucleotide
gacccagatatattagtgattgg

SEQ ID NO: 150 - DNA, 23 bp, Artificial Sequence
  Synthetic oligonucleotide
ccaatcactaatatatctgggtc

SEQ ID NO: 151 - DNA, 29 bp, Artificial Sequence
  Synthetic oligonucleotide
ctggctcttcctggtagtcaaggttgcac

SEQ ID NO: 152 - DNA, 28 bp, Artificial Sequence
  Synthetic oligonucleotide
gagccagattcctacatcagtgagaagc

SEQ ID NO: 153 - DNA, 28 bp, Artificial Sequence
  Synthetic oligonucleotide
gcttctcactgatgtaggaatctggctc

SEQ ID NO: 154 - DNA, 21 bp, Artificial Sequence
  Synthetic oligonucleotide
tcctgcatcactgagaagctc

SEQ ID NO: 155 - DNA, 21 bp, Artificial Sequence
  Synthetic oligonucleotide
gagcttctcagtgatgcagga

SEQ ID NO: 156 - DNA, 22 bp, Artificial Sequence
  Synthetic oligonucleotide
ctgcatcagtaagaagctcttc

SEQ ID NO: 157 - DNA, 22 bp, Artificial Sequence
  Synthetic oligonucleotide
gaagagcttcttactgatgcag

SEQ ID NO: 158 - DNA, 22 bp, Artificial Sequence
  Synthetic oligonucleotide
ctgcatcagtgggaagctcttc

SEQ ID NO: 159 - DNA, 22 bp, Artificial Sequence
  Synthetic oligonucleotide
gaagagcttcccactgatgcag

SEQ ID NO: 160 - DNA, 20 bp, Artificial Sequence
  Synthetic oligonucleotide
cagtgagaagttcttcatgg

SEQ ID NO: 161 - DNA, 20 bp, Artificial Sequence
  Synthetic oligonucleotide
ccaggaagaacttctcactg

SEQ ID NO: 162 - DNA, 29 bp, Artificial Sequence
  Synthetic oligonucleotide
gcatcagtgagaagttcttcatggagatg

SEQ ID NO: 163 - DNA, 29 bp, Artificial Sequence
  Synthetic oligonucleotide
catctccatgaagaacttctcactgatgc

SEQ ID NO: 164 - DNA, 22 bp, Artificial Sequence
  Synthetic oligonucleotide
cttcatggagagggcagagctc

SEQ ID NO: 165 - DNA, 22 bp, Artificial Sequence
  Synthetic oligonucleotide
gagctctgccctctccatgaag

SEQ ID NO: 166 - DNA, 22 bp, Artificial Sequence
  Synthetic oligonucleotide
cttcatggagatagcagagctc

SEQ ID NO: 167 - DNA, 22 bp, Artificial Sequence
  Synthetic oligonucleotide
gagctctgctatctccatgaag

SEQ ID NO: 168 - DNA, 22 bp, Artificial Sequence
  Synthetic oligonucleotide
catggagatggtagagctcatg

SEQ ID NO: 169 - DNA, 22 bp, Artificial Sequence
  Synthetic oligonucleotide
catgagctctaccatctccatg

SEQ ID NO: 170 - DNA, 22 bp, Artificial Sequence
  Synthetic oligonucleotide
gcagagctcagggtctcagaag

SEQ ID NO: 171 - DNA, 22 bp, Artificial Sequence
  Synthetic oligonucleotide
cttctgagaccctgagctctgc

SEQ ID NO: 172 - DNA, 25 bp, Artificial Sequence
  Synthetic oligonucleotide
ctcagaaggctgtaaggatgcaggt

SEQ ID NO: 173 - DNA, 25 bp, Artificial Sequence
  Synthetic oligonucleotide
acctgcatccttacagccttctgag

SEQ ID NO: 174 - DNA, 22 bp, Artificial Sequence
  Synthetic oligonucleotide
ctcagaaggctcgaaggatgca

SEQ ID NO: 175 - DNA, 22 bp, Artificial Sequence
  Synthetic oligonucleotide
tgcatccttcgagccttctgag

SEQ ID NO: 176 - DNA, 21 bp, Artificial Sequence
  Synthetic oligonucleotide
ccagatatgtcagtgattggc

SEQ ID NO: 177 - DNA, 21 bp, Artificial Sequence
  Synthetic oligonucleotide
gccaatcactgacatatctgg

SEQ ID NO: 178 - DNA, 21 bp, Artificial Sequence
  Synthetic oligonucleotide
gatatgttagcgattggcaac

SEQ ID NO: 179 - DNA, 21 bp, Artificial Sequence
  Synthetic oligonucleotide
gttgccaatcgctaacatatc

SEQ ID NO: 180 - DNA, 23 bp, Artificial Sequence
  Synthetic oligonucleotide
cagatatgttaatgattggcaac

SEQ ID NO: 181 - DNA, 23 bp, Artificial Sequence
  Synthetic oligonucleotide
gttgccaatcattaacatatctg

SEQ ID NO: 182 - DNA, 23 bp, Artificial Sequence
  Synthetic oligonucleotide
tatgttagtgactggcaactttg

SEQ ID NO: 183 - DNA, 23 bp, Artificial Sequence
  Synthetic oligonucleotide
caaagttgccagtcactaacata

SEQ ID NO: 184 - DNA, 19 bp, Artificial Sequence
  Synthetic oligonucleotide
ttagtgattgtcaactttg

SEQ ID NO: 185 - DNA, 19 bp, Artificial Sequence
  Synthetic oligonucleotide
caaagttgacaatcactaa

SEQ ID NO: 186 - DNA, 21 bp, Artificial Sequence
  Synthetic oligonucleotide
gttagtgatttgcaactttgg

SEQ ID NO: 187 - DNA, 21 bp, Artificial Sequence
  Synthetic oligonucleotide
ccaaagttgcaaatcactaac

SEQ ID NO: 188 - DNA, 23 bp, Artificial Sequence
  Synthetic oligonucleotide
tgttagtgattagcaactttggc

SEQ ID NO: 189 - DNA, 23 bp, Artificial Sequence
  Synthetic oligonucleotide
gccaaagttgctaatcactaaca

SEQ ID NO: 190 - DNA, 23 bp, Artificial Sequence
  Synthetic oligonucleotide
gtgattggcaaatttggcctcag

SEQ ID NO: 191 - DNA, 23 bp, Artificial Sequence
  Synthetic oligonucleotide
ctgaggccaaatttgccaatcac

SEQ ID NO: 192 - DNA, 21 bp, Artificial Sequence
  Synthetic oligonucleotide
gtgattggcagctttggcctc

SEQ ID NO: 193 - DNA, 21 bp, Artificial Sequence
  Synthetic oligonucleotide
gaggccaaagctgccaatcac

SEQ ID NO: 194 - DNA, 25 bp, Artificial Sequence
  Synthetic oligonucleotide
caactttggcctcggctggaatcag

SEQ ID NO: 195 - DNA, 25 bp, Artificial Sequence
  Synthetic oligonucleotide
ctgattccagccgaggccaaagttg

SEQ ID NO: 196 - DNA, 23 bp, Artificial Sequence
  Synthetic oligonucleotide
ctttggcctcaactggaatcagc

SEQ ID NO: 197 - DNA, 23 bp, Artificial Sequence
  Synthetic oligonucleotide
gctgattccagttgaggccaaag

SEQ ID NO: 198 - DNA, 22 bp, Artificial Sequence
  Synthetic oligonucleotide
agctggaatcggcaagtaactc

SEQ ID NO: 199 - DNA, 22 bp, Artificial Sequence
  Synthetic oligonucleotide
gagttacttgccgattccagct

SEQ ID NO: 200 - DNA, 23 bp, Artificial Sequence
  Synthetic oligonucleotide
cagctggaatcaccaagtaactc

SEQ ID NO: 201 - DNA, 22 bp, Artificial Sequence
  Synthetic oligonucleotide
gaaggatgcagattatgagtac

SEQ ID NO: 202 - DNA, 22 bp, Artificial Sequence
  Synthetic oligonucleotide
gtactcataatctgcatccttc

SEQ ID NO: 203 - DNA, 25 bp, Artificial Sequence
  Synthetic oligonucleotide
ggatgcaggttgtgagtacctctgc

SEQ ID NO: 204 - DNA, 25 bp, Artificial Sequence
  Synthetic oligonucleotide
gcagaggtactcacaacctgcatcc

SEQ ID NO: 205 - DNA, 22 bp, Artificial Sequence
  Synthetic oligonucleotide
ggttatgaggacctctgcattg

SEQ ID NO: 206 - DNA, 22 bp, Artificial Sequence
  Synthetic oligonucleotide
caatgcagaggtcctcataacc

SEQ ID NO: 207 - DNA, 24 bp, Artificial Sequence
  Synthetic oligonucleotide
gttatgagtaccsctgcattgatg

SEQ ID NO: 208 - DNA, 24 bp, Artificial Sequence
  Synthetic oligonucleotide
catcaatgcagsggtactcataac

SEQ ID NO: 209 - DNA, 21 bp, Artificial Sequence
  Synthetic oligonucleotide
cctctgcatthatgactgttg

SEQ ID NO: 210 - DNA, 21 bp, Artificial Sequence
  Synthetic oligonucleotide
caacagtcatdaatgcagagg

SEQ ID NO: 211 - DNA, 27 bp, Artificial Sequence
  Synthetic oligonucleotide
tacctctgcattaatgactgttggatg

SEQ ID NO: 212 - DNA, 27 bp, Artificial Sequence
  Synthetic oligonucleotide
catccaacagtcattaatgcagaggta

SEQ ID NO: 213 - DNA, 27 bp, Artificial Sequence
  Synthetic oligonucleotide
tacctctgcattcatgactgttggatg

SEQ ID NO: 214 - DNA, 27 bp, Artificial Sequence
  Synthetic oligonucleotide
catccaacagtcatgaatgcagaggta

SEQ ID NO: 215 - DNA, 34 bp, Artificial Sequence
  Synthetic oligonucleotide
gagtacctctgcatttatgactgttggatggctc

SEQ ID NO: 216 - DNA, 34 bp, Artificial Sequence
  Synthetic oligonucleotide
gagccatccaacagtcataaatgcagaggtactc

SEQ ID NO: 217 - DNA, 22 bp, Artificial Sequence
  Synthetic oligonucleotide
ctgcattgatggctgttggatg

SEQ ID NO: 218 - DNA, 22 bp, Artificial Sequence
  Synthetic oligonucleotide
catccaacagccatcaatgcag

SEQ ID NO: 219 - DNA, 22 bp, Artificial Sequence
  Synthetic oligonucleotide
ctgcattgatgtctgttggatg

SEQ ID NO: 220 - DNA, 22 bp, Artificial Sequence
  Synthetic oligonucleotide
catccaacagacatcaatgcag

SEQ ID NO: 221 - DNA, 22 bp, Artificial Sequence
  Synthetic oligonucleotide
ctgcattgataactgttggatg

SEQ ID NO: 222 - DNA, 22 bp, Artificial Sequence
  Synthetic oligonucleotide
catccaacagttatcaatgcag

SEQ ID NO: 223 - DNA, 24 bp, Artificial Sequence
  Synthetic oligonucleotide
gcattgatgactcttggatggctc

SEQ ID NO: 224 - DNA, 24 bp, Artificial Sequence
  Synthetic oligonucleotide
gagccatccaagagtcatcaatgc

SEQ ID NO: 225 - DNA, 23 bp, Artificial Sequence
  Synthetic oligonucleotide
gagttacttggtgattccagctg

SEQ ID NO: 226 - DNA, 21 bp, Artificial Sequence
  Synthetic oligonucleotide
cagctggaataagcaagtaac

SEQ ID NO: 227 - DNA, 21 bp, Artificial Sequence
  Synthetic oligonucleotide
gttacttgcttattccagctg

SEQ ID NO: 228 - DNA, 21 bp, Artificial Sequence
  Synthetic oligonucleotide
ggaatcagcatgtaactcaga

SEQ ID NO: 229 - DNA, 21 bp, Artificial Sequence
  Synthetic oligonucleotide
tctgagttacatgctgattcc

SEQ ID NO: 230 - DNA, 22 bp, Artificial Sequence
  Synthetic oligonucleotide
ctggaatcagaaagtaactcag

SEQ ID NO: 231 - DNA, 21 bp, Artificial Sequence
  Synthetic oligonucleotide
ctgagttactttctgattcca

SEQ ID NO: 232 - DNA, 21 bp, Artificial Sequence
  Synthetic oligonucleotide
cagcaagtaaatcagatggcc

SEQ ID NO: 233 - DNA, 21 bp, Artificial Sequence
  Synthetic oligonucleotide
ggccatctgatttacttgctg

SEQ ID NO: 234 - DNA, 21 bp, Artificial Sequence
  Synthetic oligonucleotide
caagtaactccgatggccctc

SEQ ID NO: 235 - DNA, 21 bp, Artificial Sequence
  Synthetic oligonucleotide
gagggccatcggagttacttg

SEQ ID NO: 236 - DNA, 20 bp, Artificial Sequence
  Synthetic oligonucleotide
gtaactcagacggccctctg

SEQ ID NO: 237 - DNA, 20 bp, Artificial Sequence
  Synthetic oligonucleotide
cagagggccgtctgagttac

SEQ ID NO: 238 - DNA, 23 bp, Artificial Sequence
  Synthetic oligonucleotide
taactcagatgcccctctgggct

SEQ ID NO: 239 - DNA, 23 bp, Artificial Sequence
  Synthetic oligonucleotide
agcccagaggggcatctgagtta

SEQ ID NO: 240 - DNA, 22 bp, Artificial Sequence
  Synthetic oligonucleotide
aactcagatggacctctgggct

SEQ ID NO: 241 - DNA, 22 bp, Artificial Sequence
  Synthetic oligonucleotide
agcccagaggtccatctgagtt

SEQ ID NO: 242 - DNA, 21 bp, Artificial Sequence
  Synthetic oligonucleotide
gatggccctcggggctatcat

SEQ ID NO: 243 - DNA, 21 bp, Artificial Sequence
  Synthetic oligonucleotide
atgatagccccgagggccatc

SEQ ID NO: 244 - DNA, 21 bp, Artificial Sequence
  Synthetic oligonucleotide
atggccctctgtgctatcatg

SEQ ID NO: 245 - DNA, 21 bp, Artificial Sequence
  Synthetic oligonucleotide
catgatagcacagagggccat

SEQ ID NO: 246 - DNA, 22 bp, Artificial Sequence
  Synthetic oligonucleotide
gccctctgggatatcatggctg

SEQ ID NO: 247 - DNA, 22 bp, Artificial Sequence
  Synthetic oligonucleotide
cagccatgatatcccagagggc

SEQ ID NO: 248 - DNA, 19 bp, Artificial Sequence
  Synthetic oligonucleotide
gccctctggcctatcatgg

SEQ ID NO: 249 - DNA, 24 bp, Artificial Sequence
  Synthetic oligonucleotide
gcattgatgactattggatggctc

SEQ ID NO: 250 - DNA, 24 bp, Artificial Sequence
  Synthetic oligonucleotide
gagccatccaatagtcatcaatgc

SEQ ID NO: 251 - DNA, 21 bp, Artificial Sequence
  Synthetic oligonucleotide
gatgactgttcgatggctccc

SEQ ID NO: 252 - DNA, 21 bp, Artificial Sequence
  Synthetic oligonucleotide
gggagccatcgaacagtcatc

SEQ ID NO: 253 - DNA, 23 bp, Artificial Sequence
  Synthetic oligonucleotide
ctgttggatgcctccccaaagag

SEQ ID NO: 254 - DNA, 23 bp, Artificial Sequence
  Synthetic oligonucleotide
ctctttggggaggcatccaacag

SEQ ID NO: 255 - DNA, 22 bp, Artificial Sequence
  Synthetic oligonucleotide
gctccccaaamagattcagaag

SEQ ID NO: 256 - DNA, 22 bp, Artificial Sequence
  Synthetic oligonucleotide
cttctgaatctktttggggagc

SEQ ID NO: 257 - DNA, 24 bp, Artificial Sequence
  Synthetic oligonucleotide
ggctccccaaacagattcagaagg

SEQ ID NO: 258 - DNA, 24 bp, Artificial Sequence
  Synthetic oligonucleotide
ccttctgaatctgtttggggagcc

SEQ ID NO: 259 - DNA, 25 bp, Artificial Sequence
  Synthetic oligonucleotide
caaagagattcacaaggcagacttc

SEQ ID NO: 260 - DNA, 25 bp, Artificial Sequence
  Synthetic oligonucleotide
gaagtctgccttgtgaatctctttg

SEQ ID NO: 261 - DNA, 25 bp, Artificial Sequence
  Synthetic oligonucleotide
gcagaccctcagagctttcctcatg

SEQ ID NO: 262 - DNA, 25 bp, Artificial Sequence
  Synthetic oligonucleotide
catgaggaaagctctgagggtctgc

SEQ ID NO: 263 - DNA, 24 bp, Artificial Sequence
  Synthetic oligonucleotide
cagaccctcagtgctttcctcatg

SEQ ID NO: 264 - DNA, 24 bp, Artificial Sequence
  Synthetic oligonucleotide
catgaggaaagcactgagggtctg

SEQ ID NO: 265 - DNA, 20 bp, Artificial Sequence
  Synthetic oligonucleotide
ccctcagcgctctcctcatg

SEQ ID NO: 266 - DNA, 20 bp, Artificial Sequence
  Synthetic oligonucleotide
catgaggagagcgctgaggg

SEQ ID NO: 267 - DNA, 22 bp, Artificial Sequence
  Synthetic oligonucleotide
ctcatgggatttgccagctagc

SEQ ID NO: 268 - DNA, 22 bp, Artificial Sequence
  Synthetic oligonucleotide
gctagctggcaaatcccatgag

SEQ ID NO: 269 - DNA, 23 bp, Artificial Sequence
  Synthetic oligonucleotide
gattcgccagccagctaattatg

SEQ ID NO: 270 - DNA, 23 bp, Artificial Sequence
  Synthetic oligonucleotide
cataattagctggctggcgaatc

SEQ ID NO: 271 - DNA, 28 bp, Artificial Sequence
  Synthetic oligonucleotide
tcgccagctamctaattatgttcacagc

SEQ ID NO: 272 - DNA, 28 bp, Artificial Sequence
  Synthetic oligonucleotide
gctgtgaacataattagktagctggcga

SEQ ID NO: 273 - DNA, 29 bp, Artificial Sequence
  Synthetic oligonucleotide
gctagctaattatgatcacagcaaaggac

SEQ ID NO: 274 - DNA, 19 bp, Artificial Sequence
  Synthetic oligonucleotide
ccatgataggccagagggc

SEQ ID NO: 275 - DNA, 25 bp, Artificial Sequence
  Synthetic oligonucleotide
ctctgggctttcatggctgctcctt

SEQ ID NO: 276 - DNA, 25 bp, Artificial Sequence
  Synthetic oligonucleotide
aaggagcagccatgaaagcccagag

SEQ ID NO: 277 - DNA, 21 bp, Artificial Sequence
  Synthetic oligonucleotide
gggctatcatcgctgctcctt

SEQ ID NO: 278 - DNA, 21 bp, Artificial Sequence
  Synthetic oligonucleotide
aaggagcagcgatgatagccc

SEQ ID NO: 279 - DNA, 23 bp, Artificial Sequence
  Synthetic oligonucleotide
ctatcatggctcctcctttattc

SEQ ID NO: 280 - DNA, 23 bp, Artificial Sequence
  Synthetic oligonucleotide
gaataaaggaggagccatgatag

SEQ ID NO: 281 - DNA, 22 bp, Artificial Sequence
  Synthetic oligonucleotide
catggctgctgctttattcatg

SEQ ID NO: 282 - DNA, 22 bp, Artificial Sequence
  Synthetic oligonucleotide
catgaataaagcagcagccatg

SEQ ID NO: 283 - DNA, 22 bp, Artificial Sequence
  Synthetic oligonucleotide
catggctgctwctttattcatg

SEQ ID NO: 284 - DNA, 22 bp, Artificial Sequence
  Synthetic oligonucleotide
catgaataaagwagcagccatg

SEQ ID NO: 285 - DNA, 28 bp, Artificial Sequence
  Synthetic oligonucleotide
gctgctcctttatgcatgtctaatgacc

SEQ ID NO: 286 - DNA, 28 bp, Artificial Sequence
  Synthetic oligonucleotide
ggtcattagacatgcataaaggagcagc

SEQ ID NO: 287 - DNA, 25 bp, Artificial Sequence
  Synthetic oligonucleotide
ctttattcatgtktaatgacctccg

SEQ ID NO: 288 - DNA, 25 bp, Artificial Sequence
  Synthetic oligonucleotide
cggaggtcattamacatgaataaag

SEQ ID NO: 289 - DNA, 23 bp, Artificial Sequence
  Synthetic oligonucleotide
attcatgtctagtgacctccgac

SEQ ID NO: 290 - DNA, 23 bp, Artificial Sequence
  Synthetic oligonucleotide
gtcggaggtcactagacatgaat

SEQ ID NO: 291 - DNA, 24 bp, Artificial Sequence
  Synthetic oligonucleotide
tattcatgtctaaggacctccgac

SEQ ID NO: 292 - DNA, 24 bp, Artificial Sequence
  Synthetic oligonucleotide
gtcggaggtccttagacatgaata

SEQ ID NO: 293 - DNA, 24 bp, Artificial Sequence
  Synthetic oligonucleotide
tattcatgtctcatgacctccgac

SEQ ID NO: 294 - DNA, 24 bp, Artificial Sequence
  Synthetic oligonucleotide
gtcggaggtcatgagacatgaata

SEQ ID NO: 295 - DNA, 26 bp, Artificial Sequence
  Synthetic oligonucleotide
tcatgtctaatggcctccgacacatc

SEQ ID NO: 296 - DNA, 26 bp, Artificial Sequence
  Synthetic oligonucleotide
gatgtgtcggaggccattagacatga

SEQ ID NO: 297 - DNA, 24 bp, Artificial Sequence
  Synthetic oligonucleotide
gtctaatgacccccgacacatcag

SEQ ID NO: 298 - DNA, 24 bp, Artificial Sequence
  Synthetic oligonucleotide
ctgatgtgtcgggggtcattagac

SEQ ID NO: 299 - DNA, 29 bp, Artificial Sequence
  Synthetic oligonucleotide
gtcctttgctgtgatcataattagctagc

SEQ ID NO: 300 - DNA, 22 bp, Artificial Sequence
  Synthetic oligonucleotide
cacagcaaagaactgaagctag

SEQ ID NO: 301 - DNA, 22 bp, Artificial Sequence
  Synthetic oligonucleotide
ctagcttcagttctttgctgtg

SEQ ID NO: 302 - DNA, 21 bp, Artificial Sequence
  Synthetic oligonucleotide
cagcaaaggaccgaagctagg

SEQ ID NO: 303 - DNA, 24 bp, Artificial Sequence
  Synthetic oligonucleotide
atccctagcttcggtcctttgctg

SEQ ID NO: 304 - DNA, 24 bp, Artificial Sequence
  Synthetic oligonucleotide
aggactgaagccagggatttatgc

SEQ ID NO: 305 - DNA, 24 bp, Artificial Sequence
  Synthetic oligonucleotide
gcataaatccctggcttcagtcct

SEQ ID NO: 306 - DNA, 28 bp, Artificial Sequence
  Synthetic oligonucleotide
ggactgaagctagagatttatgcagatg

SEQ ID NO: 307 - DNA, 28 bp, Artificial Sequence
  Synthetic oligonucleotide
catctgcataaatctctagcttcagtcc

SEQ ID NO: 308 - DNA, 27 bp, Artificial Sequence
  Synthetic oligonucleotide
gactgaagctaaggatttatgcagatg

SEQ ID NO: 309 - DNA, 27 bp, Artificial Sequence
  Synthetic oligonucleotide
catctgcataaatccttagcttcagtc

SEQ ID NO: 310 - DNA, 24 bp, Artificial Sequence
  Synthetic oligonucleotide
gctagggatttctgcagatgttgg

SEQ ID NO: 311 - DNA, 24 bp, Artificial Sequence
  Synthetic oligonucleotide
ccaacatctgcagaaatccctagc

SEQ ID NO: 312 - DNA, 25 bp, Artificial Sequence
  Synthetic oligonucleotide
gctagggatttatgtagatgttgga

SEQ ID NO: 313 - DNA, 25 bp, Artificial Sequence
  Synthetic oligonucleotide
tccaacatctacataaatccctagc

SEQ ID NO: 314 - DNA, 21 bp, Artificial Sequence
  Synthetic oligonucleotide
ggatttatgcacatgttggaa

SEQ ID NO: 315 - DNA, 21 bp, Artificial Sequence
  Synthetic oligonucleotide
ttccaacatgtgcataaatcc

SEQ ID NO: 316 - DNA, 30 bp, Artificial Sequence
  Synthetic oligonucleotide
gggatttatgcacatgttggaaataaaacc

SEQ ID NO: 317 - DNA, 30 bp, Artificial Sequence
  Synthetic oligonucleotide
ggttttatttccaacatgtgcataaatccc

SEQ ID NO: 318 - DNA, 24 bp, Artificial Sequence
  Synthetic oligonucleotide
tgcagatgttgaaaataaaacctg

SEQ ID NO: 319 - DNA, 24 bp, Artificial Sequence
  Synthetic oligonucleotide
caggttttattttcaacatctgca

SEQ ID NO: 320 - DNA, 24 bp, Artificial Sequence
  Synthetic oligonucleotide
tgcagatgttagaaataaaacctg

SEQ ID NO: 321 - DNA, 24 bp, Artificial Sequence
  Synthetic oligonucleotide
caggttttatttctaacatctgca

SEQ ID NO: 322 - DNA, 37 bp, Artificial Sequence
  Synthetic oligonucleotide
ggatttatgcagatgttgaaaataaaacctgcgcagc

SEQ ID NO: 323 - DNA, 37 bp, Artificial Sequence
  Synthetic oligonucleotide
gctgcgcaggttttattttcaacatctgcataaatcc

SEQ ID NO: 324 - DNA, 22 bp, Artificial Sequence
  Synthetic oligonucleotide
gtctaatgacttccgacacatc

SEQ ID NO: 325 - DNA, 22 bp, Artificial Sequence
  Synthetic oligonucleotide
gatgtgtcggaagtcattagac

SEQ ID NO: 326 - DNA, 22 bp, Artificial Sequence
  Synthetic oligonucleotide
gtctaatgaccaccgacacatc

SEQ ID NO: 327 - DNA, 22 bp, Artificial Sequence
  Synthetic oligonucleotide
gatgtgtcggtggtcattagac

SEQ ID NO: 328 - DNA, 23 bp, Artificial Sequence
  Synthetic oligonucleotide
ctaatgacctcggacacatcagc

SEQ ID NO: 329 - DNA, 23 bp, Artificial Sequence
  Synthetic oligonucleotide
gctgatgtgtccgaggtcattag

SEQ ID NO: 330 - DNA, 23 bp, Artificial Sequence
  Synthetic oligonucleotide
ctaatgacctcccacacatcagc

SEQ ID NO: 331 - DNA, 23 bp, Artificial Sequence
  Synthetic oligonucleotide
gctgatgtgtgggaggtcattag

SEQ ID NO: 332 - DNA, 23 bp, Artificial Sequence
  Synthetic oligonucleotide
ctccgacacaacagccctcaagc

SEQ ID NO: 333 - DNA, 23 bp, Artificial Sequence
  Synthetic oligonucleotide
gcttgagggctgttgtgtcggag

SEQ ID NO: 334 - DNA, 20 bp, Artificial Sequence
  Synthetic oligonucleotide
gccaaagctttccttcagga

SEQ ID NO: 335 - DNA, 20 bp, Artificial Sequence
  Synthetic oligonucleotide
tcctgaaggaaagctttggc

SEQ ID NO: 336 - DNA, 22 bp, Artificial Sequence
  Synthetic oligonucleotide
gctctccttcacgataaggacg

SEQ ID NO: 337 - DNA, 22 bp, Artificial Sequence
  Synthetic oligonucleotide
cgtccttatcgtgaaggagagc

SEQ ID NO: 338 - DNA, 21 bp, Artificial Sequence
  Synthetic oligonucleotide
ctctccttcagtataaggacg

SEQ ID NO: 339 - DNA, 21 bp, Artificial Sequence
  Synthetic oligonucleotide
cgtccttatactgaaggagag

SEQ ID NO: 340 - DNA, 21 bp, Artificial Sequence
  Synthetic oligonucleotide
gataaggacgaaattgccatc

SEQ ID NO: 341 - DNA, 21 bp, Artificial Sequence
  Synthetic oligonucleotide
gatggcaatttcgtccttatc

SEQ ID NO: 342 - DNA, 22 bp, Artificial Sequence
  Synthetic oligonucleotide
aaggacgtaamtgccatcaatc

SEQ ID NO: 343 - DNA, 22 bp, Artificial Sequence
  Synthetic oligonucleotide
gattgatggcakttacgtcctt

SEQ ID NO: 344 - DNA, 22 bp, Artificial Sequence
  Synthetic oligonucleotide
aattgccatcattcaggacccc

SEQ ID NO: 345 - DNA, 22 bp, Artificial Sequence
  Synthetic oligonucleotide
ggggtcctgaatgatggcaatt

SEQ ID NO: 346 - DNA, 22 bp, Artificial Sequence
  Synthetic oligonucleotide
aattgccatcaagcaggacccc

SEQ ID NO: 347 - DNA, 22 bp, Artificial Sequence
  Synthetic oligonucleotide
ggggtcctgcttgatggcaatt

SEQ ID NO: 348 - DNA, 22 bp, Artificial Sequence
  Synthetic oligonucleotide
aattgccatctatcaggacccc

SEQ ID NO: 349 - DNA, 37 bp, Artificial Sequence
  Synthetic oligonucleotide
ggatttatgcagatgttcgaaataaaacctgcgcagc

SEQ ID NO: 350 - DNA, 37 bp, Artificial Sequence; identical to SEQ ID NO: 349
  Synthetic oligonucleotide

SEQ ID NO: 351 - DNA, 22 bp, Artificial Sequence
  Synthetic oligonucleotide
ggaaataaaatctgcgcaggct

SEQ ID NO: 352 - DNA, 22 bp, Artificial Sequence
  Synthetic oligonucleotide
agcctgcgcagattttatttcc

SEQ ID NO: 353 - DNA, 24 bp, Artificial Sequence
  Synthetic oligonucleotide
ggaaataaaacccgcgcaggcttc

SEQ ID NO: 354 - DNA, 24 bp, Artificial Sequence
  Synthetic oligonucleotide
gaagcctgcgcgggttttatttcc

SEQ ID NO: 355 - DNA, 24 bp, Artificial Sequence
  Synthetic oligonucleotide
gaaataaaacctrcgcaggcttcc

SEQ ID NO: 356 - DNA, 24 bp, Artificial Sequence
  Synthetic oligonucleotide
ggaagcctgcgyaggttttatttc

SEQ ID NO: 357 - DNA, 28 bp, Artificial Sequence
  Synthetic oligonucleotide
ggaaataaaacctgggcaggcttccctg

SEQ ID NO: 358 - DNA, 28 bp, Artificial Sequence
  Synthetic oligonucleotide
cagggaagcctgcccaggttttatttcc

SEQ ID NO: 359 - DNA, 25 bp, Artificial Sequence
  Synthetic oligonucleotide
gaaataaaacctgcacaggcttccc

SEQ ID NO: 360 - DNA, 25 bp, Artificial Sequence
  Synthetic oligonucleotide
gggaagcctgtgcaggttttatttc

SEQ ID NO: 361 - DNA, 22 bp, Artificial Sequence
  Synthetic oligonucleotide
ataaaacctgcccaggcttccc

SEQ ID NO: 362 - DNA, 22 bp, Artificial Sequence
  Synthetic oligonucleotide
gggaagcctgggcaggttttat

SEQ ID NO: 363 - DNA, 19 bp, Artificial Sequence
  Synthetic oligonucleotide
cctgcgcagtcttccctgg

SEQ ID NO: 364 - DNA, 19 bp, Artificial Sequence
  Synthetic oligonucleotide
ccagggaagactgcgcagg

SEQ ID NO: 365 - DNA, 20 bp, Artificial Sequence
  Synthetic oligonucleotide
ggcttccctaggagttttgg

SEQ ID NO: 366 - DNA, 20 bp, Artificial Sequence
  Synthetic oligonucleotide
ccaaaactcctagggaagcc

SEQ ID NO: 367 - DNA, 21 bp, Artificial Sequence
  Synthetic oligonucleotide
ttccctgggaattttggatac

SEQ ID NO: 368 - DNA, 21 bp, Artificial Sequence
  Synthetic oligonucleotide
gtatccaaaattcccagggaa

SEQ ID NO: 369 - DNA, 20 bp, Artificial Sequence
  Synthetic oligonucleotide
ccctgggaggtttggatact

SEQ ID NO: 370 - DNA, 20 bp, Artificial Sequence
  Synthetic oligonucleotide
agtatccaaacctcccaggg

SEQ ID NO: 371 - DNA, 24 bp, Artificial Sequence
  Synthetic oligonucleotide
gttttggatactgcgacattgatg

SEQ ID NO: 372 - DNA, 24 bp, Artificial Sequence
  Synthetic oligonucleotide
catcaatgtcgcagtatccaaaac

SEQ ID NO: 373 - DNA, 22 bp, Artificial Sequence
  Synthetic oligonucleotide
ggggtcctgatagatggcaatt

SEQ ID NO: 374 - DNA, 22 bp, Artificial Sequence
  Synthetic oligonucleotide
tgccatcaatgaggaccccttg

SEQ ID NO: 375 - DNA, 22 bp, Artificial Sequence
  Synthetic oligonucleotide
caaggggtcctcattgatggca

SEQ ID NO: 376 - DNA, 22 bp, Artificial Sequence
  Synthetic oligonucleotide
tgccatcaatcgggaccccttg

SEQ ID NO: 377 - DNA, 22 bp, Artificial Sequence
  Synthetic oligonucleotide
caaggggtcccgattgatggca

SEQ ID NO: 378 - DNA, 20 bp, Artificial Sequence
  Synthetic oligonucleotide
ggaccccttggacaagcaag

SEQ ID NO: 379 - DNA, 20 bp, Artificial Sequence
  Synthetic oligonucleotide
cttgcttgtccaaggggtcc

SEQ ID NO: 380 - DNA, 22 bp, Artificial Sequence
  Synthetic oligonucleotide
cttgggcaagraagggtaccag

SEQ ID NO: 381 - DNA, 22 bp, Artificial Sequence
  Synthetic oligonucleotide
ctggtacccttycttgcccaag

SEQ ID NO: 382 - DNA, 19 bp, Artificial Sequence
  Synthetic oligonucleotide
ggcaagcaaaggtaccagc

SEQ ID NO: 383 - DNA, 19 bp, Artificial Sequence
  Synthetic oligonucleotide
gctggtacctttgcttgcc

SEQ ID NO: 384 - DNA, 19 bp, Artificial Sequence
  Synthetic oligonucleotide
ggcaagcaagygtaccagc

SEQ ID NO: 385 - DNA, 19 bp, Artificial Sequence
  Synthetic oligonucleotide
gctggtacrcttgcttgcc

SEQ ID NO: 386 - DNA, 25 bp, Artificial Sequence
  Synthetic oligonucleotide
tgggcaagcaagagtaccagcttag

SEQ ID NO: 387 - DNA, 25 bp, Artificial Sequence
  Synthetic oligonucleotide
ctaagctggtactcttgcttgccca

SEQ ID NO: 388 - DNA, 21 bp, Artificial Sequence
  Synthetic oligonucleotide
gagacaactttaaagtgtggg

SEQ ID NO: 389 - DNA, 21 bp, Artificial Sequence
  Synthetic oligonucleotide
cccacactttaaagttgtctc

SEQ ID NO: 390 - DNA, 20 bp, Artificial Sequence
  Synthetic oligonucleotide
ctttgaagtgcgggaacgac

SEQ ID NO: 391 - DNA, 20 bp, Artificial Sequence
  Synthetic oligonucleotide
gtcgttcccgcacttcaaag

SEQ ID NO: 392 - DNA, 23 bp, Artificial Sequence
  Synthetic oligonucleotide
gaagtgtgggaccgacctctctc

SEQ ID NO: 393 - DNA, 23 bp, Artificial Sequence
  Synthetic oligonucleotide
gagagaggtcggtcccacacttc

SEQ ID NO: 394 - DNA, 23 bp, Artificial Sequence
  Synthetic oligonucleotide
gaagtgtggaaacgacctctctc

SEQ ID NO: 395 - DNA, 23 bp, Artificial Sequence
  Synthetic oligonucleotide
gagagaggtcgtttccacacttc

SEQ ID NO: 396 - DNA, 22 bp, Artificial Sequence
  Synthetic oligonucleotide
gtgtgggaacaacctctctcag

SEQ ID NO: 397 - DNA, 21 bp, Artificial Sequence
  Synthetic oligonucleotide
ctacgacattcatgcccagac

SEQ ID NO: 398 - DNA, 21 bp, Artificial Sequence
  Synthetic oligonucleotide
gtctgggcatgaatgtcgtag

SEQ ID NO: 399 - DNA, 22 bp, Artificial Sequence
  Synthetic oligonucleotide
gacattgatacccagacctttg

SEQ ID NO: 400 - DNA, 22 bp, Artificial Sequence
  Synthetic oligonucleotide
caaaggtctgggtatcaatgtc

SEQ ID NO: 401 - DNA, 23 bp, Artificial Sequence
  Synthetic oligonucleotide
ctttgctgaccggggagtagatc

SEQ ID NO: 402 - DNA, 23 bp, Artificial Sequence
  Synthetic oligonucleotide
gatctactccccggtcagcaaag

SEQ ID NO: 403 - DNA, 23 bp, Artificial Sequence
  Synthetic oligonucleotide
ctttgctgactgcggagtagatc

SEQ ID NO: 404 - DNA, 23 bp, Artificial Sequence
  Synthetic oligonucleotide
gatctactccgcagtcagcaaag

SEQ ID NO: 405 - DNA, 21 bp, Artificial Sequence
  Synthetic oligonucleotide
gctgactgggtagtagatctg

SEQ ID NO: 406 - DNA, 21 bp, Artificial Sequence
  Synthetic oligonucleotide
cagatctactacccagtcagc

SEQ ID NO: 407 - DNA, 26 bp, Artificial Sequence
  Synthetic oligonucleotide
ctggggagtagttctgctaaaatttg

SEQ ID NO: 408 - DNA, 26 bp, Artificial Sequence
  Synthetic oligonucleotide
caaattttagcagaactactccccag

SEQ ID NO: 409 - DNA, 25 bp, Artificial Sequence
  Synthetic oligonucleotide
gagtagatctgccaaaatttgatgg

SEQ ID NO: 410 - DNA, 25 bp, Artificial Sequence
  Synthetic oligonucleotide
ccatcaaattttggcagatctactc

SEQ ID NO: 411 - DNA, 27 bp, Artificial Sequence
  Synthetic oligonucleotide
gtagatctgctaagatttgatggtttg

SEQ ID NO: 412 - DNA, 27 bp, Artificial Sequence
  Synthetic oligonucleotide
caaaccatcaaatcttagcagatctac

SEQ ID NO: 413 - DNA, 32 bp, Artificial Sequence
  Synthetic oligonucleotide
gtagatctgctaaaatctgatggttgttactg

SEQ ID NO: 414 - DNA, 32 bp, Artificial Sequence
  Synthetic oligonucleotide
cagtaacaaccatcagattttagcagatctac

SEQ ID NO: 415 - DNA, 24 bp, Artificial Sequence
  Synthetic oligonucleotide
gctaaaatttgttggttgttactg

SEQ ID NO: 416 - DNA, 24 bp, Artificial Sequence
  Synthetic oligonucleotide
cagtaacaaccaacaaattttagc

SEQ ID NO: 417 - DNA, 24 bp, Artificial Sequence
  Synthetic oligonucleotide
gctaaaatttcatggttgttactg

SEQ ID NO: 418 - DNA, 24 bp, Artificial Sequence
  Synthetic oligonucleotide
cagtaacaaccatgaaattttagc

SEQ ID NO: 419 - DNA, 27 bp, Artificial Sequence
  Synthetic oligonucleotide
ctaaaatttgatgattgttactgtgac

SEQ ID NO: 420 - DNA, 27 bp, Artificial Sequence
  Synthetic oligonucleotide
gtcacagtaacaatcatcaaattttag

SEQ ID NO: 421 - DNA, 27 bp, Artificial Sequence
  Synthetic oligonucleotide
ctaaaatttgatcgttgttactgtgac

SEQ ID NO: 422 - DNA, 22 bp, Artificial Sequence
  Synthetic oligonucleotide
ctgagagaggttgttcccacac

SEQ ID NO: 423 - DNA, 22 bp, Artificial Sequence
  Synthetic oligonucleotide
gaacgacctccctcaggcttag

SEQ ID NO: 424 - DNA, 22 bp, Artificial Sequence
  Synthetic oligonucleotide
ctaagcctgagggaggtcgttc

SEQ ID NO: 425 - DNA, 21 bp, Artificial Sequence
  Synthetic oligonucleotide
cgacctctcccaggcttagcc

SEQ ID NO: 426 - DNA, 21 bp, Artificial Sequence
  Synthetic oligonucleotide
ggctaagcctgggagaggtcg

SEQ ID NO: 427 - DNA, 23 bp, Artificial Sequence
  Synthetic oligonucleotide
ctcaggcttaccctgggctgtag

SEQ ID NO: 428 - DNA, 23 bp, Artificial Sequence
  Synthetic oligonucleotide
ctacagcccagggtaagcctgag

SEQ ID NO: 429 - DNA, 22 bp, Artificial Sequence
  Synthetic oligonucleotide
cttagcctggcctgtagctatg

SEQ ID NO: 430 - DNA, 22 bp, Artificial Sequence
  Synthetic oligonucleotide
catagctacaggccaggctaag

SEQ ID NO: 431 - DNA, 22 bp, Artificial Sequence
  Synthetic oligonucleotide
ctgggctgtagatatgataaac

SEQ ID NO: 432 - DNA, 22 bp, Artificial Sequence
  Synthetic oligonucleotide
gtttatcatatctacagcccag

SEQ ID NO: 433 - DNA, 22 bp, Artificial Sequence
  Synthetic oligonucleotide
gtagctatgaaaaaccggcagg

SEQ ID NO: 434 - DNA, 22 bp, Artificial Sequence
  Synthetic oligonucleotide
cctgccggtttttcatagctac

SEQ ID NO: 435 - DNA, 21 bp, Artificial Sequence
  Synthetic oligonucleotide
gctatgataaaacggcaggag

SEQ ID NO: 436 - DNA, 21 bp, Artificial Sequence
  Synthetic oligonucleotide
ctcctgccgttttatcatagc

SEQ ID NO: 437 - DNA, 24 bp, Artificial Sequence
  Synthetic oligonucleotide
gctatgataaactggcaggagatt

SEQ ID NO: 438 - DNA, 24 bp, Artificial Sequence
  Synthetic oligonucleotide
aatctcctgccagtttatcatagc

SEQ ID NO: 439 - DNA, 21 bp, Artificial Sequence
  Synthetic oligonucleotide
accggcaggsgattggtggac

SEQ ID NO: 440 - DNA, 21 bp, Artificial Sequence
  Synthetic oligonucleotide
gtccaccaatcscctgccggt

SEQ ID NO: 441 - DNA, 24 bp, Artificial Sequence
  Synthetic oligonucleotide
gataaaccggcagaagattggtgg

SEQ ID NO: 442 - DNA, 24 bp, Artificial Sequence
  Synthetic oligonucleotide
ccaccaatcttctgccggtttatc

SEQ ID NO: 443 - DNA, 29 bp, Artificial Sequence
  Synthetic oligonucleotide
gataaaccggcaggcgattggtggacctc

SEQ ID NO: 444 - DNA, 29 bp, Artificial Sequence
  Synthetic oligonucleotide
gaggtccaccaatcgcctgccggtttatc

SEQ ID NO: 445 - DNA, 23 bp, Artificial Sequence
  Synthetic oligonucleotide
ccggcaggagactggtggacctc

SEQ ID NO: 446 - DNA, 23 bp, Artificial Sequence
  Synthetic oligonucleotide
gaggtccaccagtctcctgccgg

SEQ ID NO: 447 - DNA, 27 bp, Artificial Sequence
  Synthetic oligonucleotide
gtcacagtaacaacgatcaaattttag

SEQ ID NO: 448 - DNA, 30 bp, Artificial Sequence
  Synthetic oligonucleotide
ctaaaatttgatggttwttactgtgacagt

SEQ ID NO: 449 - DNA, 30 bp, Artificial Sequence
  Synthetic oligonucleotide
actgtcacagtaawaaccatcaaattttag

SEQ ID NO: 450 - DNA, 30 bp, Artificial Sequence
  Synthetic oligonucleotide
ctaaaatttgatggttggtactgtgacagt

SEQ ID NO: 451 - DNA, 30 bp, Artificial Sequence
  Synthetic oligonucleotide
actgtcacagtaccaaccatcaaattttag

SEQ ID NO: 452 - DNA, 30 bp, Artificial Sequence
  Synthetic oligonucleotide
ctaaaatttgatggtcgttactgtgacagt

SEQ ID NO: 453 - DNA, 30 bp, Artificial Sequence
  Synthetic oligonucleotide
actgtcacagtaacgaccatcaaattttag

SEQ ID NO: 454 - DNA, 30 bp, Artificial Sequence
  Synthetic oligonucleotide
ctaaaatttgatggtggttactgtgacagt

SEQ ID NO: 455 - DNA, 30 bp, Artificial Sequence
  Synthetic oligonucleotide
actgtcacagtaaccaccatcaaattttag

SEQ ID NO: 456 - DNA, 21 bp, Artificial Sequence
  Synthetic oligonucleotide
ttggcagatgattataagcac

SEQ ID NO: 457 - DNA, 21 bp, Artificial Sequence
  Synthetic oligonucleotide
gtgcttataatcatctgccaa

SEQ ID NO: 458 - DNA, 21 bp, Artificial Sequence
  Synthetic oligonucleotide
ttggcagatagttataagcac

SEQ ID NO: 459 - DNA, 21 bp, Artificial Sequence
  Synthetic oligonucleotide
gtgcttataactatctgccaa

SEQ ID NO: 460 - DNA, 25 bp, Artificial Sequence
  Synthetic oligonucleotide
gttataagcacacgtccttggccct

SEQ ID NO: 461 - DNA, 25 bp, Artificial Sequence
  Synthetic oligonucleotide
agggccaaggacgtgtgcttataac

SEQ ID NO: 462 - DNA, 23 bp, Artificial Sequence
  Synthetic oligonucleotide
gttataagcacgtgtccttggcc

SEQ ID NO: 463 - DNA, 23 bp, Artificial Sequence
  Synthetic oligonucleotide
ggccaaggacacgtgcttataac

SEQ ID NO: 464 - DNA, 23 bp, Artificial Sequence
  Synthetic oligonucleotide
gtccttggcccagaataggactg

SEQ ID NO: 465 - DNA, 23 bp, Artificial Sequence
  Synthetic oligonucleotide
cagtcctattctgggccaaggac

SEQ ID NO: 466 - DNA, 23 bp, Artificial Sequence
  Synthetic oligonucleotide
gtccttggccccgaataggactg

SEQ ID NO: 467 - DNA, 23 bp, Artificial Sequence
  Synthetic oligonucleotide
cagtcctattcggggccaaggac

SEQ ID NO: 468 - DNA, 21 bp, Artificial Sequence
  Synthetic oligonucleotide
ctgaataggattggcagaagc

SEQ ID NO: 469 - DNA, 21 bp, Artificial Sequence
  Synthetic oligonucleotide
gcttctgccaatcctattcag

SEQ ID NO: 470 - DNA, 21 bp, Artificial Sequence
  Synthetic oligonucleotide
cagaagcattatgtactcctg

SEQ ID NO: 471 - DNA, 21 bp, Artificial Sequence
  Synthetic oligonucleotide
caggagtacataatgcttctg

SEQ ID NO: 472 - DNA, 21 bp, Artificial Sequence
  Synthetic oligonucleotide
caggagattagtggacctcgc

SEQ ID NO: 473 - DNA, 21 bp, Artificial Sequence
  Synthetic oligonucleotide
gcgaggtccactaatctcctg

SEQ ID NO: 474 - DNA, 21 bp, Artificial Sequence
  Synthetic oligonucleotide
ggagattggtagacctcgctc

SEQ ID NO: 475 - DNA, 21 bp, Artificial Sequence
  Synthetic oligonucleotide
gagcgaggtctaccaatctcc

SEQ ID NO: 476 - DNA, 24 bp, Artificial Sequence
  Synthetic oligonucleotide
gattggtggacttcgctcttatac

SEQ ID NO: 477 - DNA, 24 bp, Artificial Sequence
  Synthetic oligonucleotide
gtataagagcgaagtccaccaatc

SEQ ID NO: 478 - DNA, 20 bp, Artificial Sequence
  Synthetic oligonucleotide
ggtggacctcactcttatac

SEQ ID NO: 479 - DNA, 20 bp, Artificial Sequence
  Synthetic oligonucleotide
gtataagagtgaggtccacc

SEQ ID NO: 480 - DNA, 20 bp, Artificial Sequence
  Synthetic oligonucleotide
ggtggaccttgctcttatac

SEQ ID NO: 481 - DNA, 20 bp, Artificial Sequence
  Synthetic oligonucleotide
gtataagagcaaggtccacc

SEQ ID NO: 482 - DNA, 23 bp, Artificial Sequence
  Synthetic oligonucleotide
tgcttccctgcgtaaaggagtgg

SEQ ID NO: 483 - DNA, 23 bp, Artificial Sequence
  Synthetic oligonucleotide
ccactcctttacgcagggaagca

SEQ ID NO: 484 - DNA, 24 bp, Artificial Sequence
  Synthetic oligonucleotide
gtaaaggagtggactgtaatcctg

SEQ ID NO: 485 - DNA, 24 bp, Artificial Sequence
  Synthetic oligonucleotide
caggattacagtccactcctttac

SEQ ID NO: 486 - DNA, 24 bp, Artificial Sequence
  Synthetic oligonucleotide
aaaggagtggcctataatcctgcc

SEQ ID NO: 487 - DNA, 24 bp, Artificial Sequence
  Synthetic oligonucleotide
ggcaggattataggccactccttt

SEQ ID NO: 488 - DNA, 24 bp, Artificial Sequence
  Synthetic oligonucleotide
aaaggagtggcccgtaatcctgcc

SEQ ID NO: 489 - DNA, 24 bp, Artificial Sequence
  Synthetic oligonucleotide
ggcaggattacgggccactccttt

SEQ ID NO: 490 - DNA, 24 bp, Artificial Sequence
  Synthetic oligonucleotide
gtaatcctgcctacttcatcacac

SEQ ID NO: 491 - DNA, 24 bp, Artificial Sequence
  Synthetic oligonucleotide
gtgtgatgaagtaggcaggattac

SEQ ID NO: 492 - DNA, 26 bp, Artificial Sequence
  Synthetic oligonucleotide
ctgcctgcttcaacacacagctcctc

SEQ ID NO: 493 - DNA, 26 bp, Artificial Sequence
  Synthetic oligonucleotide
gaggagctgtgtgttgaagcaggcag

SEQ ID NO: 494 - DNA, 24 bp, Artificial Sequence
  Synthetic oligonucleotide
cctgcttcatcccacagctcctcc

SEQ ID NO: 495 - DNA, 24 bp, Artificial Sequence
  Synthetic oligonucleotide
ggaggagctgtgggatgaagcagg

SEQ ID NO: 496 - DNA, 24 bp, Artificial Sequence
  Synthetic oligonucleotide
cttcatcacaccgctcctccctgt

SEQ ID NO: 497 - DNA, 22 bp, Artificial Sequence
  Synthetic oligonucleotide
cattgtgtacttctgtgagtgg

SEQ ID NO: 498 - DNA, 22 bp, Artificial Sequence
  Synthetic oligonucleotide
ccactcacagaagtacacaatg

SEQ ID NO: 499 - DNA, 23 bp, Artificial Sequence
  Synthetic oligonucleotide
cattgtgtactactgtgagtggc

SEQ ID NO: 500 - DNA, 23 bp, Artificial Sequence
  Synthetic oligonucleotide
gccactcacagtagtacacaatg

SEQ ID NO: 501 - DNA, 22 bp, Artificial Sequence
  Synthetic oligonucleotide
gtgtactcctatgagtggcctc

SEQ ID NO: 502 - DNA, 22 bp, Artificial Sequence
  Synthetic oligonucleotide
gaggccactcataggagtacac

SEQ ID NO: 503 - DNA, 23 bp, Artificial Sequence
  Synthetic oligonucleotide
gtgtactcctgggagtggcctct

SEQ ID NO: 504 - DNA, 23 bp, Artificial Sequence
  Synthetic oligonucleotide
agaggccactcccaggagtacac

SEQ ID NO: 505 - DNA, 22 bp, Artificial Sequence
  Synthetic oligonucleotide
ctgtgagtggactctttatatg

SEQ ID NO: 506 - DNA, 22 bp, Artificial Sequence
  Synthetic oligonucleotide
catataaagagtccactcacag

SEQ ID NO: 507 - DNA, 22 bp, Artificial Sequence
  Synthetic oligonucleotide
ctgtgagtggcktctttatatg

SEQ ID NO: 508 - DNA, 22 bp, Artificial Sequence
  Synthetic oligonucleotide
catataaagamgccactcacag

SEQ ID NO: 509 - DNA, 21 bp, Artificial Sequence
  Synthetic oligonucleotide
tggcctctttctatgtggccc

SEQ ID NO: 510 - DNA, 21 bp, Artificial Sequence
  Synthetic oligonucleotide
gggccacatagaaagaggcca

SEQ ID NO: 511 - DNA, 25 bp, Artificial Sequence
  Synthetic oligonucleotide
agtggcctctttgtatgtggccctt

SEQ ID NO: 512 - DNA, 25 bp, Artificial Sequence
  Synthetic oligonucleotide
aagggccacatacaaagaggccact

SEQ ID NO: 513 - DNA, 35 bp, Artificial Sequence
  Synthetic oligonucleotide
cctttcaaaagcccaatgatacagaaatccgacag

SEQ ID NO: 514 - DNA, 35 bp, Artificial Sequence
  Synthetic oligonucleotide
ctgtcggatttctgtatcattgggcttttgaaagg

SEQ ID NO: 515 - DNA, 28 bp, Artificial Sequence
  Synthetic oligonucleotide
caattatacagaaaaccgacagtactgc

SEQ ID NO: 516 - DNA, 28 bp, Artificial Sequence
  Synthetic oligonucleotide
gcagtactgtcggttttctgtataattg

SEQ ID NO: 517 - DNA, 21 bp, Artificial Sequence
  Synthetic oligonucleotide
cgacagtacsgcaatcactgg

SEQ ID NO: 518 - DNA, 21 bp, Artificial Sequence
  Synthetic oligonucleotide
ccagtgattgcsgtactgtcg

SEQ ID NO: 519 - DNA, 21 bp, Artificial Sequence
  Synthetic oligonucleotide
cgacagtactacaatcactgg

SEQ ID NO: 520 - DNA, 24 bp, Artificial Sequence
  Synthetic oligonucleotide
acagggaggagcggtgtgatgaag

SEQ ID NO: 521 - DNA, 28 bp, Artificial Sequence
  Synthetic oligonucleotide
cacagctcctccgtgtgaaaaggaagct

SEQ ID NO: 522 - DNA, 28 bp, Artificial Sequence
  Synthetic oligonucleotide
agcttccttttcacacggaggagctgtg

SEQ ID NO: 523 - DNA, 23 bp, Artificial Sequence
  Synthetic oligonucleotide
ggaagctagggtactatgaatgg

SEQ ID NO: 524 - DNA, 23 bp, Artificial Sequence
  Synthetic oligonucleotide
ccattcatagtaccctagcttcc

SEQ ID NO: 525 - DNA, 22 bp, Artificial Sequence
  Synthetic oligonucleotide
agggttctataaatggacttca

SEQ ID NO: 526 - DNA, 22 bp, Artificial Sequence
  Synthetic oligonucleotide
tgaagtccatttatagaaccct

SEQ ID NO: 527 - DNA, 22 bp, Artificial Sequence
  Synthetic oligonucleotide
gacttcaaggtcaagaagtcac

SEQ ID NO: 528 - DNA, 22 bp, Artificial Sequence
  Synthetic oligonucleotide
gtgacttcttgaccttgaagtc

SEQ ID NO: 529 - DNA, 21 bp, Artificial Sequence
  Synthetic oligonucleotide
gaagtcacaaaaatcccacag

SEQ ID NO: 530 - DNA, 21 bp, Artificial Sequence
  Synthetic oligonucleotide
ctgtgggatttttgtgacttc

SEQ ID NO: 531 - DNA, 24 bp, Artificial Sequence
  Synthetic oligonucleotide
gtcacataaatdccacaggcactg

SEQ ID NO: 532 - DNA, 24 bp, Artificial Sequence
  Synthetic oligonucleotide
cagtgcctgtgghatttatgtgac

SEQ ID NO: 533 - DNA, 22 bp, Artificial Sequence
  Synthetic oligonucleotide
cacataaatcccaaaggcactg

SEQ ID NO: 534 - DNA, 22 bp, Artificial Sequence
  Synthetic oligonucleotide
cagtgcctttgggatttatgtg

SEQ ID NO: 535 - DNA, 22 bp, Artificial Sequence
  Synthetic oligonucleotide
cacataaatcccgcaggcactg

SEQ ID NO: 536 - DNA, 22 bp, Artificial Sequence
  Synthetic oligonucleotide
cagtgcctgcgggatttatgtg

SEQ ID NO: 537 - DNA, 21 bp, Artificial Sequence
  Synthetic oligonucleotide
atcccacagacactgttttgc

SEQ ID NO: 538 - DNA, 21 bp, Artificial Sequence
  Synthetic oligonucleotide
gcaaaacagtgtctgtgggat

SEQ ID NO: 539 - DNA, 22 bp, Artificial Sequence
  Synthetic oligonucleotide
ggcactgtttcgcttcagctag

SEQ ID NO: 540 - DNA, 22 bp, Artificial Sequence
  Synthetic oligonucleotide
ctagctgaagcgaaacagtgcc

SEQ ID NO: 541 - DNA, 29 bp, Artificial Sequence
  Synthetic oligonucleotide
gcgcttcgcttcctggacatccctggggc

SEQ ID NO: 542 - DNA, 29 bp, Artificial Sequence
  Synthetic oligonucleotide
gccccagggatgtccaggaagcgaagcgc

SEQ ID NO: 543 - DNA, 21 bp, Artificial Sequence
  Synthetic oligonucleotide
ccagtgattgtagtactgtcg

SEQ ID NO: 544 - DNA, 21 bp, Artificial Sequence
  Synthetic oligonucleotide
cagtactgcagtcactggcga

SEQ ID NO: 545 - DNA, 21 bp, Artificial Sequence
  Synthetic oligonucleotide
tcgccagtgactgcagtactg

SEQ ID NO: 546 - DNA, 19 bp, Artificial Sequence
  Synthetic oligonucleotide
cagtactgcgatcactggc

SEQ ID NO: 547 - DNA, 19 bp, Artificial Sequence
  Synthetic oligonucleotide
gccagtgatcgcagtactg

SEQ ID NO: 548 - DNA, 21 bp, Artificial Sequence
  Synthetic oligonucleotide
tactgcaatcgctggcgaaat

SEQ ID NO: 549 - DNA, 21 bp, Artificial Sequence
  Synthetic oligonucleotide
atttcgccagcgattgcagta

SEQ ID NO: 550 - DNA, 17 bp, Artificial Sequence
  Synthetic oligonucleotide
gcaatcaccggcgaaat

SEQ ID NO: 551 - DNA, 17 bp, Artificial Sequence
  Synthetic oligonucleotide
atttcgccggtgattgc

SEQ ID NO: 552 - DNA, 22 bp, Artificial Sequence
  Synthetic oligonucleotide
gcaatcactgtcgaaattttgc

SEQ ID NO: 553 - DNA, 22 bp, Artificial Sequence
  Synthetic oligonucleotide
gcaaaatttcgacagtgattgc

SEQ ID NO: 554 - DNA, 26 bp, Artificial Sequence
  Synthetic oligonucleotide
gcaatcactggcaaaattttgctgac

SEQ ID NO: 555 - DNA, 31 bp, Artificial Sequence
  Synthetic oligonucleotide
gcagaccctcagcgccagctagctaattatg

SEQ ID NO: 556 - DNA, 31 bp, Artificial Sequence
  Synthetic oligonucleotide
cataattagctagctggcgctgagggtctgc

SEQ ID NO: 557 - DNA, 26 bp, Artificial Sequence
  Synthetic oligonucleotide
gttttggatactacattgatgcccag

SEQ ID NO: 558 - DNA, 26 bp, Artificial Sequence
  Synthetic oligonucleotide
ctgggcatcaatgtagtatccaaaac

SEQ ID NO: 559 - DNA, 24 bp, Artificial Sequence
  Synthetic oligonucleotide
ctcctgtgagtggatgtggccctt

SEQ ID NO: 560 - DNA, 24 bp, Artificial Sequence
  Synthetic oligonucleotide
aagggccacatccactcacaggag

SEQ ID NO: 561 - DNA, 23 bp, Artificial Sequence
  Synthetic oligonucleotide
caggagagaattgatgttgctgg

SEQ ID NO: 562 - DNA, 23 bp, Artificial Sequence
  Synthetic oligonucleotide
ccagcaacatcaattctctcctg

SEQ ID NO: 563 - DNA, 25 bp, Artificial Sequence
  Synthetic oligonucleotide
gataaaccggcagattggtggacct

SEQ ID NO: 564 - DNA, 25 bp, Artificial Sequence
  Synthetic oligonucleotide
aggtccaccaatctgccggtttatc

SEQ ID NO: 565 - DNA, 35 bp, Artificial Sequence
  Synthetic oligonucleotide
gactggacatcttggacatcttttaaccaggagag

SEQ ID NO: 566 - DNA, 35 bp, Artificial Sequence
  Synthetic oligonucleotide
ctctcctggttaaaagatgtccaagatgtccagtc